European Patent Application EP 4 335 448 A1, published March 13, 2024. Title: Modified oncolytic parvovirus H-1PV with an enchanced fitness and superior anticancer activity. Applicant: Deutsches Krebsforschungszentrum. Application EP. The sequence listing filed with the application follows.

SEQUENCE LISTING (5 sequences)

SEQ ID NO: 1 - DNA, 21 bp, synthetic construct
  source 1..21: mol_type = other DNA
tcaatgcgctcaccatctctg

SEQ ID NO: 2 - DNA, 21 bp, synthetic construct
  source 1..21: mol_type = other DNA
ttagtccaaggtcagctcctc

SEQ ID NO: 3 - DNA, 29 bp, synthetic construct
  source 1..29: mol_type = other DNA
taatatggtattggttaactgtaaaaaat

SEQ ID NO: 4 - DNA, 20 bp, synthetic construct
  source 1..20: mol_type = other DNA
caaccacccaaccacccttt

SEQ ID NO: 5 - DNA, 5176 bp, Mus musculus
  source 1..5176: mol_type = genomic DNA
catttttagaactgaccaaccatgttcacgcaagtgacgtgatgacgcgcgctgcgcgcgctgccttcggcagtcacacgtcactagcgtttcacatggttggtcagttctaaaaatgataagcggttcagagagtttgaaaccaaggcgggaaacggaagtgggcgtggctaactgtatataagcagtcactctggtcggttactcactctgctttcatttctgagtttgtgagacacaggagcgagactaaccaactaaccatggctggaaacgcttactccgatgaggttttgggagtaacaaactggctgaaggacaaaagtagccaggaggtgttctcatttgtttttaaaaatgaaaacgtccaactaaatggaaaggacatcggttggaatagttacagaaaggagctacaagatgacgagctgaagtctctacaacgaggggcggagaccacttgggaccaaagcgaggacatggaatgggagagcgcagtggatgacatgaccaaaaagcaagtatttatttttgattctttggttaagaagtgtttgtttgaagtgctcagcacaaagaacatagctcctagtaatgttacttggttcgtgcagcatgaatggggaaaggacccaggctggcactgtcatgtgctgattggaggcaaggactttagtcaacctcaaggaaaatggtggagaaggcagctaaatgtgtactggagtagatggttggtgactgcctgtaatgttcaactaacaccagctgaaagaattaaactgagagaaatagcagaggacagtgaatgggtcactttgcttacctataagcataagcacaccaagaaggactataccaagtgtgttctttttggaaacatgattgcttattactttttaagcaaaaagaaaatatgtaccagtccaccaagggacggaggctattttcttagcagtgactctggctggaaaactaactttttgaaagagggcgagcgccatctagtgagcaaactgtatactgatgagatgaaaccagaaacggtcgagaccacagtgaccactgcacaggaagctaagcgcggcagaattcaaactagagaggaggtctcgattaaaaccacactcaaagagttggtacataaaagagtaacctcaccagaagactggatgatgatgcagccagacagttacattgaaatgatggctcaaccaggtggagaaaacttgcttaaaaatacactagagatctgtacactgactctagcaagaaccaaaacagcctttgacttgattctggaaaaagctgaaaccagcaaactagccaacttttccatggctagcaccagaacctgtagaatctttgctgagcatggctggaactatattaaagtctgccatgccatctgttgtgtgctgaatagacaaggaggcaaaaggaacactgtgctctttcacggaccagccagcacaggcaaatctattattgcacaagccatagcacaagcagttggtaatgttggttgttacaatgctgccaatgtgaactttccatttaatgactgtaccaacaaaaacttgatttgggtggaagaagctggtaactttggccagcaagtaaaccaattcaaagctatttgttctggccaaaccatacgcattgatcaaaaaggaaaaggcagcaaacagattgaaccaacaccagttattatgaccaccaacgagaacattaccgtggttagaataggctgtgaggaaagaccagaacacactcaaccaatcagagacagaatgctcaacattcacctgacacgtacactacctggtgactttggtttggtggataagcacgaatggcctctgatctgtgcttggttggtgaagaatggttaccaatctaccatggcttgttactgtgctaaatggggcaaagttcctgattggtcagaggactgggcggagccgaagctagacactcctataaattcgctaggttcaatgcgctcaccatctctgactccgagaagtacgcctctcagccaaaactacgctcttactccacttgcatcggaccttgcggacctagctctagagccttggagcacaccaaatactcctgttgcgggcactgcagcaagccaaaacactggggaggctggttccacagcctgccaaggtgctcaacggagcccaacctggtccgagatcgaggcggatttgagagcttgcttcagtcaagaacagttggagagcgacttcaacgaggagctgaccttggactaaggtacaatggcacctccagctaaaagagctaaaagaggtaaggggctaagggatggttggttggtggggtactaatgtatgactacctgttttacaggcctgaaatcacttggttctaggttgggtgcctcctggctacaagtacctgggaccagggaacagccttgaccaaggagaaccaaccaacccttctgacgccgctgccaaagaacacgacgaagcctacgaccaatacatcaaatctggaaaaaatccttacctgtacttctctcctgctgatcaacgcttcattgaccaaaccaaagacgccaaggactggggcggcaaggttggtcactacttttttagaaccaagcgagcttttgcacctaagctttctactgactctgaacctggcacttctggtgtgagcagacctggtaaacgaactaaaccacctgctcacatttttgtaaatcaagccagagctaaaaaaaaacgcgcttctcttgctgcacagcagaggactctgacaatgagtgatggcaccgaaacaaaccaaccagacactggaatcgctaatgctagagttgagcgatcagctgacggaggtggaagctctgggggtgggggctctggcgggggtgggattggtgtttctactgggacttatgataatcaaacgacttataagtttttgggagatggatgggtagaaataactgcacatgcttctagacttttgcacttgggaatgcctccttcagaaaactactgccgcgtcaccgttcacaataatcaaacaacaggacacggaactaaggtaaagggaaacatggcctatgacacacatcaacaaatttggacaccatggagcttggtagatgctaatgcttggggagtttggttccaaccaagtgactggcagttcattcaaaacagcatggaatcgctgaatcttgactcattgagccaagaactatttaatgtagtagtcaaaacagtcactgaacaacaaggagctggccaagatgccattaaagtctataataatgacttgacggcctgtatgatggttgctctggatagtaacaacatactgccttacacacctgcagctcaaacatcagaaacacttggtttctacccatggaaaccaaccgcaccagctccttacagatactactttttcatgcctagacaactcagtgtaacctctagcaactctgctgaaggaactcaaatcacagacaccattggagagccacaggcactaaactctcaattttttactattgagaacaccttgcctattactctcctgcgcacaggtgatgagtttacaactggcacctacatctttaacactgacccacttaaacttactcacacatggcaaaccaacagacacttggcatgcctccaaggaataactgacctaccaacatcagatacagcaacagcatcactaactgcaaatggagacagatttggatcaacacaaacacagaatgtgaactatgtcacagaggctttgcgcaccaggcctgctcagattggcttcatgcaacctcatgacaactttgaagcaaacagaggtggcccatttaaggttccagtggtaccgctagacataacagctggcgaggaccatgatgcaaacggagccatacgatttaactatggcaaacaacatggcgaagattgggccaaacaaggagcagcaccagaaaggtacacatgggatgcaattgatagtgcagctgggagggacacagctagatgctttgtacaaagtgcaccaatatctattccaccaaaccaaaaccagatcttgcagcgagaagacgccatagctggcagaactaacatgcattatactaatgtttttaacagctatggtccacttagtgcatttcctcatccagatcccatttatccaaatggacaaatttgggacaaagaattggacctggaacacaaacctagactacacgtaactgcaccatttgtttgtaaaaacaacccaccaggtcaactatttgttcacttggggcctaatctgactgaccaatttgacccaaacagcacaactgtttctcgcattgttacatatagcactttttactggaagggtattttgaaattcaaagccaaactaagaccaaatctgacctggaatcctgtataccaagcaaccacagactctgttgccaattcttacatgaatgttaagaaatggctcccatctgcaactggcaacatgcactctgatccattgatttgtagacctgtgcctcacatgacatactaaccaaccaactatgtttctctgtttgcttcacataatacttaaactaactagactacaacataaaaatatacacttaataatagattattaaaaataacataatatggtaggttaactgtaaaaaataatagaacttttggaataaatatagttagttggttaatgttagatagaatataaaaagattttgtattttaaaataaatatagttagttggttaatgttagatagaatataaaaagattttgtatttgggaaataaaaagggtggttgggtggttggttggtactcccttagactgaatgttagggaccaaaaaaataataaaataattaaaatgaacaaggactactgtctattcagttgaccaactgaacctatagtatcactatgtttttagggtgggggggtgggagatacatacgttcgctatggaccaagtggtaccggttggttgctaagctcgaacaagacggctaagccggtccggttggttgagcgcaaccaaccggtaccacttggtccatagcgaacgtatgtatctcccacccccccaccctaaaaacatagtgatactataggttcagttggtcaactgaa